European Patent Specification EP 3 517 609 B1, published May 1, 2024. Title: Improved recombinant Fc gamma RII. Applicant: Sagami Chemical Research Institute TOSOH Corporation. The sequence listing filed with the application follows.

SEQUENCE LISTING (176 sequences)

SEQ ID NO: 1 - protein, 209 aa, Artificial Sequence
  MalE signal - FcgRIIb - 6His
MKIKTGARILALSALTTMMFSASALAMGTPAAPPKAVLKLEPQWINVLQEDSVTLTCRGTHSPESDSIQWFHNGNLIPTHTQPSYRFKANNNDSGEYTCQTGQTSLSDPVHLTVLSEWLVLQTPHLEFQEGETIVLRCHSWKDKPLVKVTFFQNGKSKKFSRSDPNFSIPQANHSHSGDYHCTGNIGYTLYSSKPVTITVQGGHHHHHH

SEQ ID NO: 2 - protein, 209 aa, Artificial Sequence
  MalE signal - FcgRIIb-a4F3 - 6His
MKIKTGARILALSALTTMMFSASALAMGTPAAPPKAVLKLEPQWINVLQEDSVTLTCRGTHSPESDSIQWFHNGNLIPTHTQPTYRFKANNNDSGEYTCQTGQTSLSDPVHLTVLSEWLVLQTPHLEFQEGETIVLRCHSWKDKPLVKVTFFQNGKSKKFSRSDPNFSIPQANHSHSGDYHCTGNIGYTLYSSKPVTITVQGGHHHHHH

SEQ ID NO: 3 - protein, 209 aa, Artificial Sequence
  MalE signal - FcgRIIb-a2E2 - 6His
MKIKTGARILALSALTTMMFSASALAMGTPAAPPKAVLKLEPQWINVLQEDSVTLTCRGTHSPESDSIQWFHNGNLIPTHTQPSYRFKANNNDSGEYTCQTGQTSLSDPVHLTVLSEWLVLQTPRLEFQEGETIVLRCHSWKDKPLVKVTFFQNGKSKKFSRSDPNFSIPQANHSHSGDYHCTGNIGYTLYSSKPVTITVQGGHHHHHH

SEQ ID NO: 4 - protein, 209 aa, Artificial Sequence
  MalE signal - FcgRIIb-a15A6 - 6His
MKIKTGARILALSALTTMMFSASALAMGTPAAPPKAVLKLEPQWINVLQEDSVTLTCRGTHSPESDSVQWFHNGNLIPTHTQPSYRFKANNNDSGEYTCQTGQTSLSDPVHLTVLSEWLVLQTPHLEFQEGETIVLRCHSWKDKPLVKVTFFQNGKSKKFSRSDPNFSIPQANHSHSGDYHCTGNIGYTLYSSKPVTITVQGGHHHHHH

SEQ ID NO: 5 - protein, 209 aa, Artificial Sequence
  MalE signal - FcgRIIb-m3 - 6His
MKIKTGARILALSALTTMMFSASALAMGTPAAPPKAVLKLEPQWINVLQEDSVTLTCRGTHSPESDSVQWFHNGNLIPTHTQPTYRFKANNNDSGEYTCQTGQTSLSDPVHLTVLSEWLVLQTPRLEFQEGETIVLRCHSWKDKPLVKVTFFQNGKSKKFSRSDPNFSIPQANHSHSGDYHCTGNIGYTLYSSKPVTITVQGGHHHHHH

SEQ ID NO: 6 - protein, 209 aa, Artificial Sequence
  MalE signal - FcgRIIb-d10D5 - 6His
MKIKTGARILALSALTTMMFSASALAMGTPAAPPKAVLKLEPQWINVLQEDSVTLTCRGTHSPESDSVQWFHNGNLIPTHTQPTYRFKANSNDSGEYTCQTGQTSLSDPVHLTVLSEWLVLQTPRLEFQEGETIVLRCHSWKDKPLVKVTFFQNGKSKKFSRSDPNFSIPQANHSHSGDYHCTGNIGYTLYSSKPVTITVQGGHHHHHH

SEQ ID NO: 7 - protein, 209 aa, Artificial Sequence
  MalE signal - FcgRIIb-d11D7 - 6His
MKIKTGARILALSALTTMMFSASALAMGTPAAPPKAVLKLEPQWINVLQEDSVTLTCRGTHSPESDSVQWFHNGNLIPTHTQPTYRFKATNNDSGEYTCQTGQTSLSDPVHLTVLSEWLVLQTPRLEFQEGETIVLRCHSWKDKPLVKVTFFQNGKSKKFSRSDPNFSIPQANHSHSGDYHCTGNIGYTLYSSKPVTITVQGGHHHHHH

SEQ ID NO: 8 - protein, 209 aa, Artificial Sequence
  MalE signal - FcgRIIb-d6E2 - 6His
MKIKTGARILALSALTTMMFSASALAMGTPAAPPKAVLKLEPQWINVLQEDSVTLTCRGTHSPESDSVQWFHNGNLIPTQTQPTYRFKANNNDSGEYTCQTGQTSLSDPVHLTVLSEWLVLQTPRLEFQEGETIVLRCHSWKDKPLVKVTFFQNGKSKKFSRSDPNFSIPQANHSHSGDYHCTGNIGYTLYSSKPVTITVQGGHHHHHH

SEQ ID NO: 9 - protein, 209 aa, Artificial Sequence
  MalE signal - FcgRIIb-m5b - 6His
MKIKTGARILALSALTTMMFSASALAMGTPAAPPKAVLKLEPQWINVLQEDSVTLTCRGTHSPESDSVQWFHNGNLIPTQTQPTYRFKANSNDSGEYTCQTGQTSLSDPVHLTVLSEWLVLQTPRLEFQEGETIVLRCHSWKDKPLVKVTFFQNGKSKKFSRSDPNFSIPQANHSHSGDYHCTGNIGYTLYSSKPVTITVQGGHHHHHH

SEQ ID NO: 10 - protein, 209 aa, Artificial Sequence
  MalE signal - FcgRIIb-m5c - 6His
MKIKTGARILALSALTTMMFSASALAMGTPAAPPKAVLKLEPQWINVLQEDSVTLTCRGTHSPESDSVQWFHNGNLIPTHTQPTYRFKATSNDSGEYTCQTGQTSLSDPVHLTVLSEWLVLQTPRLEFQEGETIVLRCHSWKDKPLVKVTFFQNGKSKKFSRSDPNFSIPQANHSHSGDYHCTGNIGYTLYSSKPVTITVQGGHHHHHH

SEQ ID NO: 11 - protein, 209 aa, Artificial Sequence
  MalE signal - FcgRIIb-m6b - 6His
MKIKTGARILALSALTTMMFSASALAMGTPAAPPKAVLKLEPQWINVLQEDSVTLTCRGTHSPESDSVQWFHNGNLIPTQTQPTYRFKATSNDSGEYTCQTGQTSLSDPVHLTVLSEWLVLQTPRLEFQEGETIVLRCHSWKDKPLVKVTFFQNGKSKKFSRSDPNFSIPQANHSHSGDYHCTGNIGYTLYSSKPVTITVQGGHHHHHH

SEQ ID NO: 12 - protein, 310 aa, Homo sapiens
  ref <308>: UniProt P31994
  ref <309>: 2000-05-30
  ref <313>: (1)..(310)
MGILSFLPVLATESDWADCKSPQPWGHMLLWTAVLFLAPVAGTPAAPPKAVLKLEPQWINVLQEDSVTLTCRGTHSPESDSIQWFHNGNLIPTHTQPSYRFKANNNDSGEYTCQTGQTSLSDPVHLTVLSEWLVLQTPHLEFQEGETIVLRCHSWKDKPLVKVTFFQNGKSKKFSRSDPNFSIPQANHSHSGDYHCTGNIGYTLYSSKPVTITVQAPSSSPMGIIVAVVTGIAVAAIVAAVVALIYCRKKRISALPGYPECREMGETLPEKPANPTNPDEADKVGAENTITYSLLMHPDALEEPDDQNRI

SEQ ID NO: 13 - DNA, 627 bp, Artificial Sequence
  DNA encoding MalE signal - FcgRIIb-a4F3 - 6His
atgaaaataaaaacaggtgcacgcatcctcgcattatccgcattaacgacgatgatgttttccgcctcggctctcgccatgggaactcccgcagcgcctccaaaggcggttctgaaactggagccgcagtggattaatgtgttgcaggaagatagcgtgacgctgacctgccgtggaacccatagcccggaatcagacagcatacagtggtttcacaacggcaatttgatccccactcatacgcagccgacgtaccgtttcaaagccaacaataacgattcgggcgaatatacctgccagacaggccagaccagcctgagcgatccagtgcacctgaccgtgctgtcagaatggctggtgctgcaaaccccgcatctggaatttcaggaaggcgaaaccatagtgctgcgttgccacagctggaaagataaaccgctggtgaaggtcacgttcttccagaacgggaagagcaagaagttctcccgtagcgacccgaattttagcatcccccaggcgaatcatagccatagcggcgattatcactgcaccgggaatattgggtatacgttgtatagcagcaagccggttactatcaccgtgcagggcggccatcatcatcatcatcat

SEQ ID NO: 14 - DNA, 627 bp, Artificial Sequence
  DNA encoding MalE signal - FcgRIIb-a2E2 - 6His
atgaaaataaaaacaggtgcacgcatcctcgcattatccgcattaacgacgatgatgttttccgcctcggctctcgccatgggaactcccgcagcgcctccaaaggcggttctgaaactggagccgcagtggattaatgtgttgcaggaagatagcgtgacgctgacctgccgtggaacccatagcccggaatcagacagcatacagtggtttcacaacggcaatttgatccccactcatacgcagccgtcgtaccgtttcaaagccaacaataacgattcgggcgaatatacctgccagacaggccagaccagcctgagcgatccagtgcacctgaccgtgctgtcagaatggctggtgctgcaaaccccgcgtctggaatttcaggaaggcgaaaccatagtgctgcgttgccacagctggaaagataaaccgctggtgaaggtcacgttcttccagaacgggaagagcaagaagttctcccgtagcgacccgaattttagcatcccccaggcgaatcatagccatagcggcgattatcactgcaccgggaatattgggtatacgttgtatagtagcaagccggttactatcaccgtgcagggcggccatcatcatcatcatcat

SEQ ID NO: 15 - DNA, 627 bp, Artificial Sequence
  DNA encoding MalE signal - FcgRIIb-a15A6 - 6His
atgaaaataaaaacaggtgcacgcatcctcgcattatccgcattaacgacgatgatgttttccgcctcggctctcgccatgggaactcccgcagcgcctccaaaggcggttctgaaactggagccgcagtggattaatgtgttgcaggaagatagcgtgacgctgacctgccgaggaacccatagcccggaatcagacagcgtacagtggtttcacaacggcaatttgatccccactcatacgcagccgtcgtaccgtttcaaagccaacaataacgattcgggcgaatatacctgccagacaggccagaccagcctgagcgatccagtgcacctgaccgtgctgtcagaatggctggtgctgcaaaccccgcatctggaatttcaggaaggcgaaaccatagtgctgcgttgccacagctggaaggataaaccgctggtgaaggtcacgttcttccagaacgggaagagcaagaagttctcccgtagcgacccgaattttagcatcccccaggcgaatcatagccatagcggcgattatcactgcaccgggaatattgggtatacgttgtatagcagcaagccggttactatcaccgtgcagggcggccatcatcatcatcatcat

SEQ ID NO: 16 - DNA, 627 bp, Artificial Sequence
  DNA encoding MalE signal - FcgRIIb-m3 - 6His
atgaaaataaaaacaggtgcacgcatcctcgcattatccgcattaacgacgatgatgttttccgcctcggctctcgccatgggaactcccgcagcgcctccaaaggcggttctgaaactggagccgcagtggattaatgtgttgcaggaagatagcgtgacgctgacctgccgtggaacccatagcccggaatcagacagcgtacagtggtttcacaacggcaatttgatccccactcatacgcagccgacgtaccgtttcaaagccaacaataacgattcgggcgaatatacctgccagacaggccagaccagcctgagcgatccagtgcacctgaccgtgctgtcagaatggctggtgctgcaaaccccgcgtctggaatttcaggaaggcgaaaccatagtgctgcgttgccacagctggaaagataaaccgctggtgaaggtcacgttcttccagaacgggaagagcaagaagttctcccgtagcgacccgaattttagcatcccccaggcgaatcatagccatagcggcgattatcactgcaccgggaatattgggtatacgttgtatagcagcaagccggttactatcaccgtgcagggcggccatcatcatcatcatcat

SEQ ID NO: 17 - DNA, 627 bp, Artificial Sequence
  DNA encoding MalE signal - FcgRIIb-m3 - 6His
atgaaaataaaaacaggtgcacgcatcctcgcattatccgcattaacgacgatgatgttttccgcctcggctctcgccatgggaactcccgcagcgcctccaaaggcggttctgaaactggagccgcagtggattaatgtgttgcaggaagatagcgtgacgctgacctgccgtggaacccatagcccggaatcagacagcgtacagtggtttcacaacggcaatttgatccccactcatacgcagccgacgtaccgtttcaaagccaacaataacgattcgggcgaatatacctgccagacaggccagaccagcctgtcggatccagtgcacctgaccgtgctgtcagaatggctggtgctgcaaaccccgcgtctggaatttcaggaaggcgaaaccatagtgctgcgttgccacagctggaaagataaaccgctggtgaaggtcacgttcttccagaacgggaagagcaagaagttctcccgtagcgacccgaattttagcatcccccaggcgaatcatagccatagcggcgattatcactgcaccgggaatattgggtatacgttgtatagcagcaagccggttactatcaccgtgcagggcggccatcatcatcatcatcat

SEQ ID NO: 18 - DNA, 627 bp, Artificial Sequence
  DNA encoding MalE signal - FcgRIIb-d10D5 - 6His
atgaaaataaaaacaggtgcacgcatcctcgcattatccgcattaacgacgatgatgttttccgcctcggctctcgccatgggaactcccgcagcgcctccaaaggcggttctgaaactggagccgcagtggattaatgtgttgcaggaagatagcgtgacgctgacctgccgtggaacccatagcccggaatcagacagcgtacagtggtttcacaacggcaatttgatccccactcatacgcagccgacgtaccgtttcaaagccaacagtaacgattcgggcgaatatacctgccagacaggccagaccagcctgtcggatccagtgcacctgaccgtgctgtcagaatggctggtgctgcaaaccccgcgtctggaatttcaggaaggcgaaaccatagtgctgcgttgccacagctggaaagataaaccgctggtgaaggtcacgttcttccagaacgggaagagcaagaagttctcccgtagcgacccgaattttagcatcccccaggcgaatcatagccatagcggcgattatcactgcaccgggaatattgggtatacgttgtatagcagcaagccggttactatcaccgtgcagggcggccatcatcatcatcatcat

SEQ ID NO: 19 - DNA, 627 bp, Artificial Sequence
  DNA encoding MalE signal - FcgRIIb-d11D7 - 6His
atgaaaataaaaacaggtgcacgcatcctcgcattatccgcattaacgacgatgatgttttccgcctcggctctcgccatgggaactcccgcagcgcctccaaaggcggttctgaaactggagccgcagtggattaatgtgttgcaggaagatagcgtgacgctgacctgccgtggaacccatagcccggaatcagacagcgtacagtggtttcacaacggcaatttgatccccactcatacgcagccgacgtatcgtttcaaagccaccaataacgattcgggcgaatatacctgccagacaggccagaccagcctgtcggatccagtgcacctgaccgtgctgtcagaatggctggtgctgcaaaccccgcgtctggaatttcaggaaggcgaaaccatagtgctgcgttgccacagctggaaagataaaccgctggtgaaggtcacgttcttccagaacgggaagagcaagaagttctcccgtagcgacccgaattttagcatcccccaggcgaatcatagccatagcggcgattatcactgcaccgggaatattgggtatacgttgtatagcagcaagccggttactatcaccgtgcagggcggccatcatcatcatcatcat

SEQ ID NO: 20 - DNA, 627 bp, Artificial Sequence
  DNA encoding MalE signal - FcgRIIb-d11D7 - 6His
atgaaaataaaaacaggtgcacgcatcctcgcattatccgcattaacgacgatgatgttttccgcctcggctctcgccatgggaactcccgcagcgcctccaaaggcggttctgaaactggagccgcagtggattaatgtgttgcaggaagatagcgtgacgctgacctgccgtggaacccatagcccggaatcagacagcgtacagtggtttcacaacggcaatttgatccccactcaaacgcagccgacgtaccgtttcaaagccaacaataacgattcgggcgaatatacctgccagacaggccagaccagcctgtcggatccagtgcacctgaccgtgctgtcagaatggctggtgctgcaaaccccgcgtctggaatttcaggaaggcgaaaccatagtgctgcgttgccacagctggaaagataaaccgctggtgaaggtcacgttcttccagaacgggaagagcaagaagttctcccgtagcgacccgaattttagcatcccccaggcgaatcatagccatagcggcgattatcactgcaccgggaatattgggtatacgttgtatagcagcaagccggttactatcaccgtgcagggcggccatcatcatcatcatcat

SEQ ID NO: 21 - DNA, 627 bp, Artificial Sequence
  DNA encoding MalE signal - FcgRIIb-m5b - 6His
atgaaaataaaaacaggtgcacgcatcctcgcattatccgcattaacgacgatgatgttttccgcctcggctctcgccatgggaactcccgcagcgcctccaaaggcggttctgaaactggagccgcagtggattaatgtgttgcaggaagatagcgtgacgctgacctgccgtggaacccatagcccggaatcagacagcgtacagtggtttcacaacggcaatttgatccccactcaaacgcagccgacgtaccgtttcaaagccaacagtaacgattcgggcgaatatacctgccagacaggccagaccagcctgtcggatccagtgcacctgaccgtgctgtcagaatggctggtgctgcaaaccccgcgtctggaatttcaggaaggcgaaaccatagtgctgcgttgccacagctggaaagataaaccgctggtgaaggtcacgttcttccagaacgggaagagcaagaagttctcccgtagcgacccgaattttagcatcccccaggcgaatcatagccatagcggcgattatcactgcaccgggaatattgggtatacgttgtatagcagcaagccggttactatcaccgtgcagggcggccatcatcatcatcatcat

SEQ ID NO: 22 - DNA, 627 bp, Artificial Sequence
  DNA encoding MalE signal - FcgRIIb-m5c - 6His
atgaaaataaaaacaggtgcacgcatcctcgcattatccgcattaacgacgatgatgttttccgcctcggctctcgccatgggaactcccgcagcgcctccaaaggcggttctgaaactggagccgcagtggattaatgtgttgcaggaagatagcgtgacgctgacctgccgtggaacccatagcccggaatcagacagcgtacagtggtttcacaacggcaatttgatccccactcatacgcagccgacgtaccgtttcaaagccaccagtaacgattcgggcgaatatacctgccagacaggccagaccagcctgtcggatccagtgcacctgaccgtgctgtcagaatggctggtgctgcaaaccccgcgtctggaatttcaggaaggcgaaaccatagtgctgcgttgccacagctggaaagataaaccgctggtgaaggtcacgttcttccagaacgggaagagcaagaagttctcccgtagcgacccgaattttagcatcccccaggcgaatcatagccatagcggcgattatcactgcaccgggaatattgggtatacgttgtatagcagcaagccggttactatcaccgtgcagggcggccatcatcatcatcatcat

SEQ ID NO: 23 - DNA, 627 bp, Artificial Sequence
  DNA encoding MalE signal - FcgRIIb-m6b - 6His
atgaaaataaaaacaggtgcacgcatcctcgcattatccgcattaacgacgatgatgttttccgcctcggctctcgccatgggaactcccgcagcgcctccaaaggcggttctgaaactggagccgcagtggattaatgtgttgcaggaagatagcgtgacgctgacctgccgtggaacccatagcccggaatcagacagcgtacagtggtttcacaacggcaatttgatccccactcaaacgcagccgacgtaccgtttcaaagccaccagtaacgattcgggcgaatatacctgccagacaggccagaccagcctgtcggatccagtgcacctgaccgtgctgtcagaatggctggtgctgcaaaccccgcgtctggaatttcaggaaggcgaaaccatagtgctgcgttgccacagctggaaagataaaccgctggtgaaggtcacgttcttccagaacgggaagagcaagaagttctcccgtagcgacccgaattttagcatcccccaggcgaatcatagccatagcggcgattatcactgcaccgggaatattgggtatacgttgtatagcagcaagccggttactatcaccgtgcagggcggccatcatcatcatcatcat

SEQ ID NO: 24 - DNA, 930 bp, Artificial Sequence
  DNA encoding FcgRIIb
atggggatattgagctttcttccggtgttagccaccgaaagcgattgggcggattgcaaaagcccccagccctggggccatatgctgctgtggacagcggtcctgtttctggctccggttgcggggactcccgcagcgcctccaaaggcggttctgaaactggagccgcagtggattaatgtgttgcaggaagatagcgtgacgctgacctgccgtggaacccatagcccggaatcagacagcatacagtggtttcacaacggcaatttgatccccactcatacgcagccgtcgtaccgtttcaaagccaacaataacgattcgggcgaatatacctgccagacaggccagaccagcctgagcgatccagtgcacctgaccgtgctgtcagaatggctggtgctgcaaaccccgcatctggaatttcaggaaggcgaaaccatagtgctgcgttgccacagctggaaagataaaccgctggtgaaggtcacgttcttccagaacgggaagagcaagaagttctcccgtagcgacccgaattttagcatcccccaggcgaatcatagccatagcggcgattatcactgcaccgggaatattgggtatacgttgtatagcagcaagccggttactatcaccgtgcaggcgccgagctcatcgccgatgggcattattgtggcggtagttaccggcatcgcggtggccgccattgtcgcggctgtggtagccctgatttactgccgcaaaaaacgtatcagtgctttaccgggttaccctgaatgccgtgaaatgggcgagaccctgcccgaaaaaccggcgaacccgaccaatcccgatgaagcggataaggtgggcgcagaaaacaccatcacctatagcctgctgatgcacccggatgcgctggaggaaccggatgatcaaaatcgtatt

SEQ ID NO: 25 - DNA, 38 bp, Artificial Sequence
  Oligonucleotide
atggggatattgagctttcttccggtgttagccaccga

SEQ ID NO: 26 - DNA, 40 bp, Artificial Sequence
  Oligonucleotide
ttttgcaatccgcccaatcgctttcggtggctaacaccgg

SEQ ID NO: 27 - DNA, 40 bp, Artificial Sequence
  Oligonucleotide
gattgggcggattgcaaaagcccccagccctggggccata

SEQ ID NO: 28 - DNA, 40 bp, Artificial Sequence
  Oligonucleotide
acaggaccgctgtccacagcagcatatggccccagggctg

SEQ ID NO: 29 - DNA, 40 bp, Artificial Sequence
  Oligonucleotide
gtggacagcggtcctgtttctggctccggttgcggggact

SEQ ID NO: 30 - DNA, 40 bp, Artificial Sequence
  Oligonucleotide
gaaccgcctttggaggcgctgcgggagtccccgcaaccgg

SEQ ID NO: 31 - DNA, 40 bp, Artificial Sequence
  Oligonucleotide
gcctccaaaggcggttctgaaactggagccgcagtggatt

SEQ ID NO: 32 - DNA, 40 bp, Artificial Sequence
  Oligonucleotide
acgctatcttcctgcaacacattaatccactgcggctcca

SEQ ID NO: 33 - DNA, 40 bp, Artificial Sequence
  Oligonucleotide
gtgttgcaggaagatagcgtgacgctgacctgccgtggaa

SEQ ID NO: 34 - DNA, 40 bp, Artificial Sequence
  Oligonucleotide
gctgtctgattccgggctatgggttccacggcaggtcagc

SEQ ID NO: 35 - DNA, 40 bp, Artificial Sequence
  Oligonucleotide
gcccggaatcagacagcatacagtggtttcacaacggcaa

SEQ ID NO: 36 - DNA, 40 bp, Artificial Sequence
  Oligonucleotide
tgcgtatgagtggggatcaaattgccgttgtgaaaccact

SEQ ID NO: 37 - DNA, 40 bp, Artificial Sequence
  Oligonucleotide
tgatccccactcatacgcagccgtcgtaccgtttcaaagc

SEQ ID NO: 38 - DNA, 40 bp, Artificial Sequence
  Oligonucleotide
tcgcccgaatcgttattgttggctttgaaacggtacgacg

SEQ ID NO: 39 - DNA, 40 bp, Artificial Sequence
  Oligonucleotide
aacaataacgattcgggcgaatatacctgccagacaggcc

SEQ ID NO: 40 - DNA, 40 bp, Artificial Sequence
  Oligonucleotide
cactggatcgctcaggctggtctggcctgtctggcaggta

SEQ ID NO: 41 - DNA, 40 bp, Artificial Sequence
  Oligonucleotide
agcctgagcgatccagtgcacctgaccgtgctgtcagaat

SEQ ID NO: 42 - DNA, 40 bp, Artificial Sequence
  Oligonucleotide
gcggggtttgcagcaccagccattctgacagcacggtcag

SEQ ID NO: 43 - DNA, 40 bp, Artificial Sequence
  Oligonucleotide
gtgctgcaaaccccgcatctggaatttcaggaaggcgaaa

SEQ ID NO: 44 - DNA, 40 bp, Artificial Sequence
  Oligonucleotide
tggcaacgcagcactatggtttcgccttcctgaaattcca

SEQ ID NO: 45 - DNA, 40 bp, Artificial Sequence
  Oligonucleotide
catagtgctgcgttgccacagctggaaagataaaccgctg

SEQ ID NO: 46 - DNA, 40 bp, Artificial Sequence
  Oligonucleotide
tggaagaacgtgaccttcaccagcggtttatctttccagc

SEQ ID NO: 47 - DNA, 40 bp, Artificial Sequence
  Oligonucleotide
gtgaaggtcacgttcttccagaacgggaagagcaagaagt

SEQ ID NO: 48 - DNA, 40 bp, Artificial Sequence
  Oligonucleotide
attcgggtcgctacgggagaacttcttgctcttcccgttc

SEQ ID NO: 49 - DNA, 40 bp, Artificial Sequence
  Oligonucleotide
cccgtagcgacccgaattttagcatcccccaggcgaatca

SEQ ID NO: 50 - DNA, 40 bp, Artificial Sequence
  Oligonucleotide
agtgataatcgccgctatggctatgattcgcctgggggat

SEQ ID NO: 51 - DNA, 40 bp, Artificial Sequence
  Oligonucleotide
ccatagcggcgattatcactgcaccgggaatattgggtat

SEQ ID NO: 52 - DNA, 40 bp, Artificial Sequence
  Oligonucleotide
ggcttgctgctatacaacgtatacccaatattcccggtgc

SEQ ID NO: 53 - DNA, 40 bp, Artificial Sequence
  Oligonucleotide
acgttgtatagcagcaagccggttactatcaccgtgcagg

SEQ ID NO: 54 - DNA, 40 bp, Artificial Sequence
  Oligonucleotide
catcggcgatgagctcggcgcctgcacggtgatagtaacc

SEQ ID NO: 55 - DNA, 40 bp, Artificial Sequence
  Oligonucleotide
cgagctcatcgccgatgggcattattgtggcggtagttac

SEQ ID NO: 56 - DNA, 40 bp, Artificial Sequence
  Oligonucleotide
gcggccaccgcgatgccggtaactaccgccacaataatgc

SEQ ID NO: 57 - DNA, 40 bp, Artificial Sequence
  Oligonucleotide
atcgcggtggccgccattgtcgcggctgtggtagccctga

SEQ ID NO: 58 - DNA, 40 bp, Artificial Sequence
  Oligonucleotide
gatacgttttttgcggcagtaaatcagggctaccacagcc

SEQ ID NO: 59 - DNA, 40 bp, Artificial Sequence
  Oligonucleotide
tactgccgcaaaaaacgtatcagtgctttaccgggttacc

SEQ ID NO: 60 - DNA, 40 bp, Artificial Sequence
  Oligonucleotide
cgcccatttcacggcattcagggtaacccggtaaagcact

SEQ ID NO: 61 - DNA, 40 bp, Artificial Sequence
  Oligonucleotide
atgccgtgaaatgggcgagaccctgcccgaaaaaccggcg

SEQ ID NO: 62 - DNA, 40 bp, Artificial Sequence
  Oligonucleotide
cgcttcatcgggattggtcgggttcgccggtttttcgggc

SEQ ID NO: 63 - DNA, 40 bp, Artificial Sequence
  Oligonucleotide
gaccaatcccgatgaagcggataaggtgggcgcagaaaac

SEQ ID NO: 64 - DNA, 40 bp, Artificial Sequence
  Oligonucleotide
atcagcaggctataggtgatggtgttttctgcgcccacct

SEQ ID NO: 65 - DNA, 40 bp, Artificial Sequence
  Oligonucleotide
catcacctatagcctgctgatgcacccggatgcgctggag

SEQ ID NO: 66 - DNA, 40 bp, Artificial Sequence
  Oligonucleotide
aatacgattttgatcatccggttcctccagcgcatccggg

SEQ ID NO: 67 - DNA, 37 bp, Artificial Sequence
  Oligonucleotide
ctagccatgggaactcccgcagcgcctccaaaggcgg

SEQ ID NO: 68 - DNA, 72 bp, Artificial Sequence
  Oligonucleotide
cccaagcttaatgatgatgatgatgatggccgccctgcacggtgatagtaaccggcttgctgctatacaacg

SEQ ID NO: 69 - DNA, 683 bp, Artificial Sequence
  pET-rhFcgRIIb sequence between XbaI and HindIII
tctagaaataattttgtttaactttaagaaggagatatacataatacatatgaaaataaaaacaggtgcacgcatcctcgcattatccgcattaacgacgatgatgttttccgcctcggctctcgccatgggaactcccgcagcgcctccaaaggcggttctgaaactggagccgcagtggattaatgtgttgcaggaagatagcgtgacgctgacctgccgtggaacccatagcccggaatcagacagcatacagtggtttcacaacggcaatttgatccccactcatacgcagccgtcgtaccgtttcaaagccaacaataacgattcgggcgaatatacctgccagacaggccagaccagcctgagcgatccagtgcacctgaccgtgctgtcagaatggctggtgctgcaaaccccgcatctggaatttcaggaaggcgaaaccatagtgctgcgttgccacagctggaaagataaaccgctggtgaaggtcacgttcttccagaacgggaagagcaagaagttctcccgtagcgacccgaattttagcatcccccaggcgaatcatagccatagcggcgattatcactgcaccgggaatattgggtatacgttgtatagcagcaagccggttactatcaccgtgcagggcggccatcatcatcatcatcattaagctt

SEQ ID NO: 70 - DNA, 20 bp, Artificial Sequence
  Oligonucleotide
taatacgactcactataggg

SEQ ID NO: 71 - DNA, 19 bp, Artificial Sequence
  Oligonucleotide
tatgctagttattgctcag

SEQ ID NO: 72 - DNA, 28 bp, Artificial Sequence
  Oligonucleotide
ttgtgaaaccactgtacgctgtctgatt

SEQ ID NO: 73 - DNA, 28 bp, Artificial Sequence
  Oligonucleotide
aatcagacagcgtacagtggtttcacaa

SEQ ID NO: 74 - DNA, 25 bp, Artificial Sequence
  Oligonucleotide
tgaaattccagacgcggggtttgca

SEQ ID NO: 75 - DNA, 25 bp, Artificial Sequence
  Oligonucleotide
tgcaaaccccgcgtctggaatttca

SEQ ID NO: 76 - DNA, 33 bp, Artificial Sequence
  Oligonucleotide
ggtcaggtgcactggatccgacaggctggtctg

SEQ ID NO: 77 - DNA, 33 bp, Artificial Sequence
  Oligonucleotide
cagaccagcctgtcggatccagtgcacctgacc

SEQ ID NO: 78 - DNA, 32 bp, Artificial Sequence
  Oligonucleotide
tacgtcggctgcgtttgagtggggatcaaatt

SEQ ID NO: 79 - DNA, 32 bp, Artificial Sequence
  Oligonucleotide
aatttgatccccactcaaacgcagccgacgta

SEQ ID NO: 80 - DNA, 35 bp, Artificial Sequence
  Oligonucleotide
tcgcccgaatcgttactggtggctttgaaacggta

SEQ ID NO: 81 - DNA, 35 bp, Artificial Sequence
  Oligonucleotide
taccgtttcaaagccaccagtaacgattcgggcga

SEQ ID NO: 82 - DNA, 37 bp, Artificial Sequence
  Oligonucleotide
tagccatgggcatgcgtaccgaagatctgccgaaagc

SEQ ID NO: 83 - DNA, 67 bp, Artificial Sequence
  Oligonucleotide
cccaagcttatccgcaggtatcgttgcggcagccctgcacggtgatagtaaccggcttgctgctata

SEQ ID NO: 84 - DNA, 19 bp, Artificial Sequence
  Oligonucleotide
tgtggtatggctgtgcagg

SEQ ID NO: 85 - DNA, 18 bp, Artificial Sequence
  Oligonucleotide
tcggcatggggtcaggtg

SEQ ID NO: 86 - protein, 205 aa, Artificial Sequence
  pTrc-m6b_Cys
MKYLLSTAAAGLLLLAAQPAMAMGTPAAPPKAVLKLEPQWINVLQEDSVTLTCRGTHSPESDSVQWFHNGNLIPTQTQPTYRFKATSNDSGEYTCQTGQTSLSDPVHLTVLSEWLVLQTPRLEFQEGETIVLRCHSWKDKPLVKVTFFQNGKSKKFSRSDPNFSIPQANHSHSGDYHCTGNIGYTLYSSKPVTITVQGCRNDTCG

SEQ ID NO: 87 - DNA, 615 bp, Artificial Sequence
  Oligonucleotide
atgaaatacctgctgtcgaccgctgctgctggtctgctgctcctcgctgcccagccggcgatggccatgggcactcccgcagcgcctccaaaggcggttctgaaactggagccgcagtggattaatgtgttgcaggaagatagcgtgacgctgacctgccgtggaacccatagcccggaatcagacagcgtacagtggtttcacaacggcaatttgatccccactcaaacgcagccgacgtaccgtttcaaagccaccagtaacgattcgggcgaatatacctgccagacaggccagaccagcctgtcggatccagtgcacctgaccgtgctgtcagaatggctggtgctgcaaaccccgcgtctggaatttcaggaaggcgaaaccatagtgctgcgttgccacagctggaaagataaaccgctggtgaaggtcacgttcttccagaacgggaagagcaagaagttctcccgtagcgacccgaattttagcatcccccaggcgaatcatagccatagcggcgattatcactgcaccgggaatattgggtatacgttgtatagcagcaagccggttactatcaccgtgcagggctgccgcaacgatacctgcgga

SEQ ID NO: 88 - protein, 209 aa, Artificial Sequence
  MalE signal - FcgRIIa - 6His
MKIKTGARILALSALTTMMFSASALAMGQAAAPPKAVLKLEPPWINVLQEDSVTLTCQGARSPESDSIQWFHNGNLIPTHTQPSYRFKANNNDSGEYTCQTGQTSLSDPVHLTVLSEWLVLQTPHLEFQEGETIMLRCHSWKDKPLVKVTFFQNGKSQKFSHLDPTFSIPQANHSHSGDYHCTGNIGYTLFSSKPVTITVQGGHHHHHH

SEQ ID NO: 89 - protein, 209 aa, Artificial Sequence
  MalE signal - FcgRIIa-m6 - 6His
MKIKTGARILALSALTTMMFSASALAMGQAAAPPKAVLKLEPPWINVLQEDSVTLTCQGARSPESDSVQWFHNGNLIPTQTQPTYRFKATSNDSGEYTCQTGQTSLSDPVHLTVLSEWLVLQTPRLEFQEGETIMLRCHSWKDKPLVKVTFFQNGKSQKFSHLDPTFSIPQANHSHSGDYHCTGNIGYTLFSSKPVTITVQGGHHHHHH

SEQ ID NO: 90 - protein, 317 aa, Homo sapiens
  ref <308>: UniProt P12318-1
  ref <309>: 2007-11-13
  ref <313>: (1)..(317)
MTMETQMSQNVCPRNLWLLQPLTVLLLLASADSQAAAPPKAVLKLEPPWINVLQEDSVTLTCQGARSPESDSIQWFHNGNLIPTHTQPSYRFKANNNDSGEYTCQTGQTSLSDPVHLTVLSEWLVLQTPHLEFQEGETIMLRCHSWKDKPLVKVTFFQNGKSQKFSHLDPTFSIPQANHSHSGDYHCTGNIGYTLFSSKPVTITVQVPSMGSSSPMGIIVAVVIATAVAAIVAAVVALIYCRKKRISANSTDPVKAAQFEPPGRQMIAIRKRQLEETNNDYETADGGYMTLNPRAPTDDDKNIYLTLPPNDHVNSNN

SEQ ID NO: 91 - DNA, 627 bp, Artificial Sequence
  DNA encoding MalE signal - FcgRIIa-m6 - 6His
atgaaaataaaaacaggtgcacgcatcctcgcattatccgcattaacgacgatgatgttttccgcctcggctctcgccatgggacaagccgcagcgcctccaaaggcggttctgaaactggagccgccgtggattaatgtgttgcaggaagatagcgtgacgctgacctgccagggagcccgtagcccggaatcagacagcgtacagtggtttcacaacggcaatttgatccccactcaaacgcagccgacgtaccgtttcaaagccaccagtaacgattcgggcgaatatacctgccagacaggccagaccagcctgtcggatccagtgcacctgaccgtgctgtcagaatggctggtgctgcaaaccccgcgtctggaatttcaggaaggcgaaaccataatgctgcgttgccacagctggaaagataaaccgctggtgaaggtcacgttcttccagaacgggaagagccagaagttctcccatctcgacccgacttttagcatcccccaggcgaatcatagccatagcggcgattatcactgcaccgggaatattgggtatacgttgtttagcagcaagccggttactatcaccgtgcagggcggccatcatcatcatcatcat

SEQ ID NO: 92 - DNA, 20 bp, Artificial Sequence
  Oligonucleotide
taatacgactcactataggg

SEQ ID NO: 93 - DNA, 26 bp, Artificial Sequence
  Oligonucleotide
acattaatccacggcggctccagttt

SEQ ID NO: 94 - DNA, 26 bp, Artificial Sequence
  Oligonucleotide
aaactggagccgccgtggattaatgt

SEQ ID NO: 95 - DNA, 37 bp, Artificial Sequence
  Oligonucleotide
taaaagtcgggtcgagatgggagaacttctggctctt

SEQ ID NO: 96 - DNA, 37 bp, Artificial Sequence
  Oligonucleotide
aagagccagaagttctcccatctcgacccgactttta

SEQ ID NO: 97 - DNA, 19 bp, Artificial Sequence
  Oligonucleotide
tatgctagttattgctcag

SEQ ID NO: 98 - DNA, 29 bp, Artificial Sequence
  Oligonucleotide
ttccgggctacgggctccctggcaggtca

SEQ ID NO: 99 - DNA, 29 bp, Artificial Sequence
  Oligonucleotide
tgacctgccagggagcccgtagcccggaa

SEQ ID NO: 100 - DNA, 31 bp, Artificial Sequence
  Oligonucleotide
aaccggcttgctgctaaacaacgtataccca

SEQ ID NO: 101 - DNA, 31 bp, Artificial Sequence
  Oligonucleotide
tgggtatacgttgtttagcagcaagccggtt

SEQ ID NO: 102 - DNA, 31 bp, Artificial Sequence
  Oligonucleotide
tcgccatgggacaagccgcagcgcctccaaa

SEQ ID NO: 103 - DNA, 27 bp, Artificial Sequence
  Oligonucleotide
tggcaacgcagcattatggtttcgcct

SEQ ID NO: 104 - DNA, 27 bp, Artificial Sequence
  Oligonucleotide
aggcgaaaccataatgctgcgttgcca

SEQ ID NO: 105 - DNA, 627 bp, Artificial Sequence
  DNA encoding MalE signal - FcgRIIa - 6His
atgaaaataaaaacaggtgcacgcatcctcgcattatccgcattaacgacgatgatgttttccgcctcggctctcgccatgggacaagccgcagcgcctccaaaggcggttctgaaactggagccgccgtggattaatgtgttgcaggaagatagcgtgacgctgacctgccagggagcccgtagcccggaatcagacagcatacagtggtttcacaacggcaatttgatccccactcatacgcagccgtcgtaccgtttcaaagccaacaataacgattcgggcgaatatacctgccagacaggccagaccagcctgagcgatccagtgcacctgaccgtgctgtcagaatggctggtgctgcaaaccccgcatctggaatttcaggaaggcgaaaccataatgctgcgttgccacagctggaaagataaaccgctggtgaaggtcacgttcttccagaacgggaagagccagaagttctcccatctcgacccgacttttagcatcccccaggcgaatcatagccatagcggcgattatcactgcaccgggaatattgggtatacgttgtttagcagcaagccggttactatcaccgtgcagggcggccatcatcatcatcatcat

SEQ ID NO: 106 - protein, 209 aa, Artificial Sequence; identical to SEQ ID NO: 1
  MalE signal - FcgRIIb - 6His

SEQ ID NO: 107 - protein, 310 aa, Homo sapiens; identical to SEQ ID NO: 12
  ref <308>: UniProt P31994
  ref <309>: 2000-05-30
  ref <313>: (1)..(310)

SEQ ID NO: 108 - DNA, 930 bp, Artificial Sequence; identical to SEQ ID NO: 24
  DNA encoding FcgRIIb

SEQ ID NO: 109 - DNA, 38 bp, Artificial Sequence; identical to SEQ ID NO: 25
  Oligonucleotide

SEQ ID NO: 110 - DNA, 40 bp, Artificial Sequence; identical to SEQ ID NO: 26
  Oligonucleotide

SEQ ID NO: 111 - DNA, 40 bp, Artificial Sequence; identical to SEQ ID NO: 27
  Oligonucleotide

SEQ ID NO: 112 - DNA, 40 bp, Artificial Sequence; identical to SEQ ID NO: 28
  Oligonucleotide

SEQ ID NO: 113 - DNA, 40 bp, Artificial Sequence; identical to SEQ ID NO: 29
  Oligonucleotide

SEQ ID NO: 114 - DNA, 40 bp, Artificial Sequence; identical to SEQ ID NO: 30
  Oligonucleotide

SEQ ID NO: 115 - DNA, 40 bp, Artificial Sequence; identical to SEQ ID NO: 31
  Oligonucleotide

SEQ ID NO: 116 - DNA, 40 bp, Artificial Sequence; identical to SEQ ID NO: 32
  Oligonucleotide

SEQ ID NO: 117 - DNA, 40 bp, Artificial Sequence; identical to SEQ ID NO: 33
  Oligonucleotide

SEQ ID NO: 118 - DNA, 40 bp, Artificial Sequence; identical to SEQ ID NO: 34
  Oligonucleotide

SEQ ID NO: 119 - DNA, 40 bp, Artificial Sequence; identical to SEQ ID NO: 35
  Oligonucleotide

SEQ ID NO: 120 - DNA, 40 bp, Artificial Sequence; identical to SEQ ID NO: 36
  Oligonucleotide

SEQ ID NO: 121 - DNA, 40 bp, Artificial Sequence; identical to SEQ ID NO: 37
  Oligonucleotide

SEQ ID NO: 122 - DNA, 40 bp, Artificial Sequence; identical to SEQ ID NO: 38
  Oligonucleotide

SEQ ID NO: 123 - DNA, 40 bp, Artificial Sequence; identical to SEQ ID NO: 39
  Oligonucleotide

SEQ ID NO: 124 - DNA, 40 bp, Artificial Sequence; identical to SEQ ID NO: 40
  Oligonucleotide

SEQ ID NO: 125 - DNA, 40 bp, Artificial Sequence; identical to SEQ ID NO: 41
  Oligonucleotide

SEQ ID NO: 126 - DNA, 40 bp, Artificial Sequence; identical to SEQ ID NO: 42
  Oligonucleotide

SEQ ID NO: 127 - DNA, 40 bp, Artificial Sequence; identical to SEQ ID NO: 43
  Oligonucleotide

SEQ ID NO: 128 - DNA, 40 bp, Artificial Sequence; identical to SEQ ID NO: 44
  Oligonucleotide

SEQ ID NO: 129 - DNA, 40 bp, Artificial Sequence; identical to SEQ ID NO: 45
  Oligonucleotide

SEQ ID NO: 130 - DNA, 40 bp, Artificial Sequence; identical to SEQ ID NO: 46
  Oligonucleotide

SEQ ID NO: 131 - DNA, 40 bp, Artificial Sequence; identical to SEQ ID NO: 47
  Oligonucleotide

SEQ ID NO: 132 - DNA, 40 bp, Artificial Sequence; identical to SEQ ID NO: 48
  Oligonucleotide

SEQ ID NO: 133 - DNA, 40 bp, Artificial Sequence; identical to SEQ ID NO: 49
  Oligonucleotide

SEQ ID NO: 134 - DNA, 40 bp, Artificial Sequence; identical to SEQ ID NO: 50
  Oligonucleotide

SEQ ID NO: 135 - DNA, 40 bp, Artificial Sequence; identical to SEQ ID NO: 51
  Oligonucleotide

SEQ ID NO: 136 - DNA, 40 bp, Artificial Sequence; identical to SEQ ID NO: 52
  Oligonucleotide

SEQ ID NO: 137 - DNA, 40 bp, Artificial Sequence; identical to SEQ ID NO: 53
  Oligonucleotide

SEQ ID NO: 138 - DNA, 40 bp, Artificial Sequence; identical to SEQ ID NO: 54
  Oligonucleotide

SEQ ID NO: 139 - DNA, 40 bp, Artificial Sequence; identical to SEQ ID NO: 55
  Oligonucleotide

SEQ ID NO: 140 - DNA, 40 bp, Artificial Sequence; identical to SEQ ID NO: 56
  Oligonucleotide

SEQ ID NO: 141 - DNA, 40 bp, Artificial Sequence; identical to SEQ ID NO: 57
  Oligonucleotide

SEQ ID NO: 142 - DNA, 40 bp, Artificial Sequence; identical to SEQ ID NO: 58
  Oligonucleotide

SEQ ID NO: 143 - DNA, 40 bp, Artificial Sequence; identical to SEQ ID NO: 59
  Oligonucleotide

SEQ ID NO: 144 - DNA, 40 bp, Artificial Sequence; identical to SEQ ID NO: 60
  Oligonucleotide

SEQ ID NO: 145 - DNA, 40 bp, Artificial Sequence; identical to SEQ ID NO: 61
  Oligonucleotide

SEQ ID NO: 146 - DNA, 40 bp, Artificial Sequence; identical to SEQ ID NO: 62
  Oligonucleotide

SEQ ID NO: 147 - DNA, 40 bp, Artificial Sequence; identical to SEQ ID NO: 63
  Oligonucleotide

SEQ ID NO: 148 - DNA, 40 bp, Artificial Sequence; identical to SEQ ID NO: 64
  Oligonucleotide

SEQ ID NO: 149 - DNA, 40 bp, Artificial Sequence; identical to SEQ ID NO: 65
  Oligonucleotide

SEQ ID NO: 150 - DNA, 40 bp, Artificial Sequence; identical to SEQ ID NO: 66
  Oligonucleotide

SEQ ID NO: 151 - DNA, 37 bp, Artificial Sequence; identical to SEQ ID NO: 67
  Oligonucleotide

SEQ ID NO: 152 - DNA, 72 bp, Artificial Sequence; identical to SEQ ID NO: 68
  Oligonucleotide

SEQ ID NO: 153 - DNA, 683 bp, Artificial Sequence; identical to SEQ ID NO: 69
  pET - rhFcgRIIb sequence between XbaI and HindIII

SEQ ID NO: 154 - protein, 209 aa, Artificial Sequence; identical to SEQ ID NO: 2
  MalE signal - FcgRIIb-a4F3 - 6His

SEQ ID NO: 155 - DNA, 627 bp, Artificial Sequence; identical to SEQ ID NO: 13
  DNA encoding MalE signal - FcgRIIb-a4F3 - 6His

SEQ ID NO: 156 - protein, 209 aa, Artificial Sequence; identical to SEQ ID NO: 5
  MalE signal - FcgRIIb-m3 - 6His

SEQ ID NO: 157 - DNA, 28 bp, Artificial Sequence
  Oligonucleotide
ttgtgaaaccactgtacgctgtctgatt

SEQ ID NO: 158 - DNA, 28 bp, Artificial Sequence
  Oligonucleotide
aatcagacagcgtacagtggtttcacaa

SEQ ID NO: 159 - DNA, 25 bp, Artificial Sequence
  Oligonucleotide
tgaaattccagacgcggggtttgca

SEQ ID NO: 160 - DNA, 25 bp, Artificial Sequence
  Oligonucleotide
tgcaaaccccgcgtctggaatttca

SEQ ID NO: 161 - DNA, 627 bp, Artificial Sequence; identical to SEQ ID NO: 16
  DNA encoding MalE signal - FcgRIIb-m3 - 6His

SEQ ID NO: 162 - DNA, 33 bp, Artificial Sequence; identical to SEQ ID NO: 76
  Oligonucleotide

SEQ ID NO: 163 - DNA, 33 bp, Artificial Sequence; identical to SEQ ID NO: 77
  Oligonucleotide

SEQ ID NO: 164 - DNA, 627 bp, Artificial Sequence; identical to SEQ ID NO: 17
  DNA encoding MalE signal - FcgRIIb-m3 - 6His

SEQ ID NO: 165 - protein, 209 aa, Artificial Sequence; identical to SEQ ID NO: 11
  MalE signal - FcgRIIb-m6b - 6His

SEQ ID NO: 166 - DNA, 35 bp, Artificial Sequence; identical to SEQ ID NO: 80
  Oligonucleotide

SEQ ID NO: 167 - DNA, 35 bp, Artificial Sequence; identical to SEQ ID NO: 81
  Oligonucleotide

SEQ ID NO: 168 - DNA, 32 bp, Artificial Sequence; identical to SEQ ID NO: 78
  Oligonucleotide

SEQ ID NO: 169 - DNA, 32 bp, Artificial Sequence; identical to SEQ ID NO: 79
  Oligonucleotide

SEQ ID NO: 170 - DNA, 627 bp, Artificial Sequence; identical to SEQ ID NO: 23
  DNA encoding MalE signal - FcgRIIb-m6b - 6His

SEQ ID NO: 171 - DNA, 37 bp, Artificial Sequence; identical to SEQ ID NO: 82
  Oligonucleotide

SEQ ID NO: 172 - DNA, 67 bp, Artificial Sequence; identical to SEQ ID NO: 83
  Oligonucleotide

SEQ ID NO: 173 - DNA, 19 bp, Artificial Sequence
  Oligonucleotide
tgtggtatggctgtgcagg

SEQ ID NO: 174 - DNA, 18 bp, Artificial Sequence
  Oligonucleotide
tcggcatggggtcaggtg

SEQ ID NO: 175 - protein, 205 aa, Artificial Sequence
  pTrc-Am6_Cys
MKYLLSTAAAGLLLLAAQPAMAMGQAAAPPKAVLKLEPPWINVLQEDSVTLTCQGARSPESDSVQWFHNGNLIPTQTQPTYRFKATSNDSGEYTCQTGQTSLSDPVHLTVLSEWLVLQTPRLEFQEGETIMLRCHSWKDKPLVKVTFFQNGKSQKFSHLDPTFSIPQANHSHSGDYHCTGNIGYTLFSSKPVTITVQGCRNDTCG

SEQ ID NO: 176 - DNA, 615 bp, Artificial Sequence
  Oligonucleotide
atgaaatacctgctgtcgaccgctgctgctggtctgctgctcctcgctgcccagccggcgatggccatgggacaagccgcagcgcctccaaaggcggttctgaaactggagccgccgtggattaatgtgttgcaggaagatagcgtgacgctgacctgccagggagcccgtagcccggaatcagacagcgtacagtggtttcacaacggcaatttgatccccactcaaacgcagccgacgtaccgtttcaaagccaccagtaacgattcgggcgaatatacctgccagacaggccagaccagcctgtcggatccagtgcacctgaccgtgctgtcagaatggctggtgctgcaaaccccgcgtctggaatttcaggaaggcgaaaccataatgctgcgttgccacagctggaaagataaaccgctggtgaaggtcacgttcttccagaacgggaagagccagaagttctcccatctcgacccgacttttagcatcccccaggcgaatcatagccatagcggcgattatcactgcaccgggaatattgggtatacgttgtttagcagcaagccggttactatcaccgtgcagggctgccgcaacgatacctgcgga